European Patent Specification EP 4 085 917 B1, published August 5, 2026. Title: ASSAY AND MEDICAMENT. Applicant: THE UNIVERSITY OF WARWICK. The sequence listing filed with the application follows.

SEQUENCE LISTING (25 sequences)

SEQ ID NO: 1 - DNA, 395 bp, Influenza virus
agcgaaagcaggtcaaatatattcaatatggaaagaataaaagaactaagaaatctaatgtcgcagtctcgcacccgcgagatactcacaaaaaccaccgtggaccatatggccataatcaagaagtacacatcaggaagacaggagaagactgaggggattcctcattctgggcaaagaggacaagagatatgggccagcactaagcatcaatgaactgagcaaccttgcgaaaggagagaaggctaatgtgctaattgggcaaggggatgtggtgttggtaatgaaacggaaacgggactctagcatacttactgacagccagacagcgaccaaaagaattcggatggccatcaattagtgtcgaatagtttaaaaacgaccttgtttctact

SEQ ID NO: 2 - DNA, 2341 bp, Influenza virus
agcgaaagcaggtcaattatattcaatatggaaagaataaaagaactaagaaatctaatgtcgcagtctcgcacccgcgagatactcacaaaaaccaccgtggaccatatggccataatcaagaagtacacatcaggaagacaggagaagaacccagcacttaggatgaaatggatgatggcaatgaaatatccaattacagcagacaagaggataacggaaatgattcctgagagaaatgagcaaggacaaactttatggagtaaaatgaatgatgccggatcagaccgagtgatggtatcacctctggctgtgacatggtggaataggaatggaccaatgacaaatacagttcattatccaaaaatctacaaaacttattttgaaagagtcgaaaggctaaagcatggaacctttggccctgtccattttagaaaccaagtcaaaatacgtcggagagttgacataaatcctggtcatgcagatctcagtgccaaggaggcacaggatgtaatcatggaagttgttttccctaacgaagtgggagccaggatactaacatcggaatcgcaactaacgataaccaaagagaagaaagaagaactccaggattgcaaaatttctcctttgatggttgcatacatgttggagagagaactggtccgcaaaacgagattcctcccagtggctggtggaacaagcagtgtgtacattgaagtgttgcatttgactcaaggaacatgctgggaacagatgtatactccaggaggggaagtgaagaatgatgatgttgatcaaagcttgattattgctgctaggaacatagtgagaagagctgcagtatcagcagacccactagcatctttattggagatgtgccacagcacacagattggtggaattaggatggtagacatccttaagcagaacccaacagaagagcaagccgtgggtatatgcaaggctgcaatgggactgagaattagctcatccttcagttttggtggattcacatttaagagaacaagcggatcatcagtcaagagagaggaagaggtgcttacgggcaatcttcaaacattgaagataagagtgcatgagggatatgaagagttcacaatggttgggagaagagcaacagccatactcagaaaagcaaccaggagattgattcagctgatagtgagtgggagagacgaacagtcgattgccgaagcaataattgtggccatggtattttcacaagaggattgtatgataaaagcagttagaggtgatctgaatttcgtcaatagggcgaatcagcgactgaatcctatgcatcaacttttaagacattttcagaaggatgcgaaagtgctttttcaaaattggggagttgaacctatcgacaatgtgatgggaatgattgggatattgcccgacatgactccaagcatcgagatgtcaatgagaggagtgagaatcagcaaaatgggtgtagatgagtactccagcacggagagggtagtggtgagcattgaccggttcttgagagtccgggaccaacgaggaaatgtactactgtctcccgaggaggtcagtgaaacacagggaacagagaaactgacaataacttactcatcgtcaatgatgtgggagattaatggtcctgaatcagtgttggtcaatacctatcaatggatcatcagaaactgggaaactgttaaaattcagtggtcccagaaccctacaatgctatacaataaaatggaatttgaaccatttcagtctttagtacctaaggccattagaggccaatacagtgggtttgtgagaactctgttccaacaaatgagggatgtgcttgggacatttgataccgcacagataataaaacttcttcccttcgcagccgctccaccaaagcaaagtagaatgcagttctcctcatttactgtgaatgtgaggggatcaggaatgagaatacttgtaaggggcaattctcctgtattcaactacaacaaggccacgaagagactcacagttctcggaaaggatgctggcactttaaccgaagacccagatgaaggcacagctggagtggagtccgctgttctgaggggattcctcattctgggcaaagaagacaggagatatgggccagcattaagcatcaatgaactgagcaaccttgcgaaaggagagaaggctaatgtgctaattgggcaaggagacgtggtgttggtaatgaaacgaaaacgggactctagcatacttactgacagccagacagcgaccaaaagaattcggatggccatcaattagtgtcgaatagtttaaaaacgaccttgtttctact

SEQ ID NO: 3 - DNA, 2341 bp, Influenza virus
agcaaaagcaggtcaattatattcagtatggaaagaataaaagaactacggaatctgatgtcgcagtctcgcactcgcgagatactgacaaaaaccacagtggaccatatggccataattaaaaagtacacatcggggagacaggaaaagaacccgtcacttaggatgaaatggatgatggcaatgaaatacccaatcactgctgacaaaaggataacagaaatggttccggagagaaatgaacaaggacaaactctatggagtaaaatgagtgatgctggatcagatcgagtgatggtatcacctttggctgtaacatggtggaatagaaatggacccgtgacaagtacggtccattacccaaaagtatacaagacttattttgacaaagtcgaaaggttaaaacatggaacctttggccctgttcattttagaaatcaagtcaagatacgcagaagagtagacataaaccctggtcatgcagacctcagtgccaaagaggcacaagatgtaattatggaagttgtttttcccaatgaagtgggagccaggatactaacatcagaatcgcaattaacaataactaaagagaaaaaagaagaactccgagattgcaaaatttctcccttgatggttgcatacatgttagagagagaacttgtacggaaaacaagatttctcccagttgctggcggaacaagcagtatatacattgaagttttacatttgactcaaggaacgtgttgggaacaaatgtacactccaggtggagaagtgaggaatgacgatattgaccaaagcctaattattgcggccaggaacatagtaagaagagccgcagtatcagcagatccactagcatctttattggagatgtgccacagcacacaaattggcgggacaaggatggtggacattcttagacagaacccaactgaagaacaagctgtggatatatgcaaggctgcaatgggattgagaatcagctcatccttcagctttggtgggtttacatttaaaagaacaagcgggtcatcagtcaaaaaagaggaagaagtgcttacaggcaatctccaaacattgaagataagagtacatgaggggtatgaggagttcacaatggtggggaaaagagcaacagctatactaagaaaagcaaccagaagattggttcagctcatagtgagtggaagagacgaacagtcaatagccgaagcaataatcgtggccatggtgttttcacaagaggattgcatgataaaagcagttagaggtgacctgaatttcgtcaacagagcaaatcagcggttgaaccccatgcatcagcttttaaggcattttcagaaagatgcgaaagtgctttttcaaaattggggaattgaacacatcgacagtgtgatgggaatgattggagtattaccagatatgactccaagcacagagatgtcaatgagaggaataagagtcagcaaaatgggtgtggatgaatactccagtacagagagggtggtggttagcattgatcggtttttgagagttcgagaccaacgtgggaatgtattattatctcctgaggaggtcagtgaaacacagggaactgagagactgacaataacttattcatcgtcgatgatgtgggagattaacggtcctgagtcggttttggtcaatacctatcaatggatcatcagaaattgggaagctgtcaaaattcaatggtctcagaatcctgcaatgttgtacaacaaaatggaatttgaaccatttcaatctttagtccccaaggccattagaagccaatacagtgggtttgtcagaactctattccaacaaatgagagacgtacttgggacatttgacaccacccagataataaagcttctcccttttgcagccgctccaccaaagcaaagcagaatgcagttctcttcactgactgtaaatgtgaggggatcagggatgagaatacttgtaaggggcaattctcctgtattcaactacaacaagaccactaaaagactaacaattctcggaaaagatgccggcactttaattgaagacccagatgaaagcacatccggagtggagtccgccgtcttgagagggtttctcattataggtaaggaagacagaagatacggaccagcattaagcatcaatgaactgagtaaccttgcaaaaggggaaaaggctaatgtgctaatcgggcaaggagacgtggtgttggtaatgaaacgaaaacgggactctagcatacttactgacagccagacagcgaccaaaagaattcggatggccatcaattaatgttgaatagtttaaaaacgaccttgtttctact

SEQ ID NO: 4 - DNA, 2341 bp, Influenza virus
agcaaaagcaggtcaattatattcagtatggaaagaataaaagaactacggaacctgatgtcgcagtctcgcactcgcgagatactaacaaaaaccacagtggaccatatggccataattaagaagtacacatcagggagacaggaaaagaacccgtcacttaggatgaaatggatgatggcaatgaaatatccaatcactgctgacaaaaggataacagaaatggttccggagagaaatgaacaaggacaaactctatggagtaaaatgagtgatgctgggtcagatcgagtgatggtatcacctttggctgtgacatggtggaatagaaatggacctgtgacaaatacggttcactatccaaaagtatacaagacttattttgacaaagtcgaaaggttaaaacatggaacctttggccctgttcattttagaaatcaagtcaagatacgccgaagagtggacataaaccctggtcatgcagacctcagtgccaaggaggcacaagatgtaattatggaagttgttttccccaatgaagtgggagccaggatactaacatcagaatcacaattaacaataaccaaagagaaaaaagaagaactccgagattgcaaaatttctcctttgatggttgcatacatgttagagagggaacttgtccgaaaaacgagatttctcccagttgctggcggaacaagcagtatatacattgaagttttacatttgactcaaggaacgtgttgggaacaaatgtacactccaggtggagaagtgaggaatgacgatgttgaccaaagcctaattattgcagccaggaacatagtgagaagagccgcagtatcagcagatccactagcatctttattggagatgtgccacagcacacaaattggcgggacaaggatggtggacattcttaggcagaacccgacggaagaacaagctgtggatatatgcaaggctgcaatgggattgagaatcagctcatccttcagctttggtgggtttacatttaaaagaacaagcgggtcatcagtcaaaagagaggaagaagtgcttacaggcaatctccaaacattgaaaataagagtacatgaggggtacgaggagttcacaatggtggggaaaagagcaacagctatactcagaaaagcaaccaggagattggttcaactcatagtgagtggaagggacgaacagtcaatagccgaagcaataatcgtggccatggtgttttcacaagaggattgcatgataaaagcagttagaggtgacctgaatttcgttaacagggcaaatcagcggttgaaccccatgcatcagcttttaaggcattttcagaaagatgcgaaggtgctttttcagaattggggaattgaacacatcgacagtgtgatgggaatggttggagtattaccagatatgactccaagcacagagatgtcaatgagaggaataagagtcagcaaaatgggcgtggatgaatactccagcacagagagggtggtggttagcattgatcggtttttgagagttcgagaccaacgtgggaatgtattattatctcctgaggaggtcagtgaaacacagggaacagagagactgacaataacttactcatcgtcaatgatgtgggagattaacggtcctgagtcggttttggtcaatacctatcaatgggtcatcagaaattgggaaactgtcaaaattcaatggtctcagaatcctgcaatgttgtacaacaaaatggaatttgaaccatttcaatctttagttcctaaggccattagaggccaatacagtggatttgtcagaactctattccaacaaatgagagatgtacttgggacatttgataccatccagataataaagcttctcccttttgcagccgctccaccaaagcaaagcagaatgcagttctcttcattgactgtaaatgtgaggggatcagggatgagaatacttgtaaggggcaattctcctgtattcaactacaacaagaccactaaaagactaacaattctcggaaaagatgccggcactttaattgaagacccagatgaaagcacatccggagtggagtccgctgtcttgagaggatttctcattctaggtaaggaagacagaagatacggaccagcattaagcatcaatgaactgagtaaccttgcaaaaggggaaaaggctaatgtgctaattgggcaaggagacgtggtgttggtaatgaaacgaaaacgggactctagcatacttactgacagccagacagcgaccaaaagaattcggatggccatcaattaatgttgaatagtttaaaaacgaccttgtttctact

SEQ ID NO: 5 - DNA, 2341 bp, Influenza virus
agcgaaagcaggcaaaccatttgaatggatgtcaatccgaccttacttttcttaaaagtgccagcacaaaatgctataagcacaactttcccttataccggagaccctccttacagccatgggacaggaacaggatacaccatggatactgtcaacaggacacatcagtactcagaaaaggcaagatggacaacaaacaccgaaactggagcaccgcaactcaacccgattgatgggccactgccagaagacaatgaaccaagtggttatgcccaaacagattgtgtattggaagcaatggctttccttgaggaatcccatcctggtatttttgaaaactcgtgtattgaaacgatggaggttgttcagcaaacacgagtagacaagctgacacaaggccgacagacctatgactggactttaaatagaaaccagcctgctgcaacagcattggccaacacaatagaagtgttcagatcaaatggcctcacggccaatgagtctggaaggctcatagacttccttaaggatgtaatggagtcaatgaaaaaagaagaaatggggatcacaactcattttcagagaaagagacgggtgagagacaatatgactaagaaaatgataacacagagaacaataggtaaaaggaaacagagattgaacaaaaggagttatctaattagagcattgaccctgaacacaatgaccaaagatgctgagagagggaagctaaaacggagagcaattgcaaccccagggatgcaaataagggggtttgtatactttgttgagacactggcaaggagtatatgtgagaaacttgaacaatcagggttgccagttggaggcaatgagaagaaagcaaagttggcaaatgttgtaaggaagatgatgaccaattctcaggacaccgaactttctttgaccatcactggagataacaccaaatggaacgaaaatcagaatcctcggatgtttttggccatgatcacatatatgaccagaaatcagcccgaatggttcagaaatgttctaagtattgctccaataatgttctcaaacaaaatggcgagactgggaaaagggtatatgtttgagagcaagagtatgaaacttagaactcaaatacctgcagaaatgctagcaagcattgatttgaaatatttcaatgattcaacaagaaagaagattgaaaaaatccgaccgctcttaatagaggggactgcatcattgagccctggaatgatgatgggcatgttcaatatgttaagcactgtattaggcgtctccatcctgaatcttggacaaaagagatacaccaagactacttactggtgggatggtcttcaatcctctgacgattttgctctgattgtgaatgcacccaatcatgaagggattcaagccggagtcgacaggttttatcgaacctgtaagctacatggaatcaatatgagcaagaaaaagtcttacataaacagaacaggtacatttgaattcacaagttttttctatcgttatgggtttgttgccaatttcagcatggagcttcccagttttggtgtgtctgggagcaacgagtcagcggacatgagtattggagttactgtcatcaaaaacaatatgataaacaatgatcttggtccagcaacagctcaaatggcccttcagttgttcatcaaagattacaggtacacgtaccgatgccatagaggtgacacacaaatacaaacccgaagatcatttgaaataaagaaactgtgggagcaaacccgttccaaagctggactgctggtctccgacggaggcccaaatttatacaacattagaaatctccacattcctgaagtctgcctaaaatgggaattgatggatgaggattaccaggggcgtttatgcaacccactgaacccatttgtcagccataaagaaattgaatcaatgaacaatgcagtgatgatgccagcacatggtccagccaaaaacatggagtatgatgctgttgcaacaacacactcctggatccccaaaagaaatcgatccatcttgaatacaagtcaaagaggagtacttgaagatgaacaaatgtaccaaaggtgctgcaatttatttgaaaaattcttccccagcagttcatacagaagaccagtcgggatatccagtatggtggaggctatggtttccagagcccgaattgatgcacggattgatttcgaatctggaaggataaagaaagaagagttcactgagatcatgaagatctgttccaccattgaagagctcagacggcaaaaatagtgaatttagcttgtccttcatgaaaaaatgccttgttcctact

SEQ ID NO: 6 - DNA, 2341 bp, Influenza virus
agcaaaagcaggcaaaccatttgaatggatgtcaatccgactctactgttcctaaaggttccagcgcaaaatgccataagcaccacattcccttatactggggatcctccatacagccatggaacaggaacagggtacaccatggacacagtcaacagaacacaccaatattcagagaaggggaagtggacgacaaatacagaaactggggcaccccaactcaacccaattgatggaccactacctgaggataatgagccaagtggatatgcacaaacagactgtgtcctggaggctatggccttccttgaagaatcccacccaggtatctttgagaactcatgccttgaaacaatggaagtcgttcaacaaacaagggtggacaaactaactcaaggtcgccagacttatgattggacattaaacagaaatcaaccagcagcaactgcattagccaacaccatagaagtttttagatcgaatggactaacagctaatgaatcaggaaggctaatagatttcctcaaggatgtgatggaatcaatggataaagaggaaatggagataacaacacactttcaaagaaaaaggagagtaagagacaacatgaccaagaaaatggtcacacaaagaacaatagggaagaaaaaacaaagagtggataagagaggctatctaataagagctttgacattgaacacgatgaccaaagatgcagagagaggtaaattaaaaagaagggctattgcaacacccgggatgcaaattagagggttcgtgtacttcgttgaaactttagctagaagcatttgcgaaaagcttgaacagtctggactcccggttgggggtaatgaaaagaaggccaaactggcaaatgttgtgagaaaaatgatgactaattcacaagacactgagctttctttcacaatcactggggacaacactaagtggaatgaaaatcaaaaccctcgaatgtttttggcgatgattacatatatcacaaaaaatcaacctgagtggttcagaaacatcctgagcatcgcaccaataatgttctcaaacaaaatggcaagactaggaaaaggatacatgttcgagagtaagaggatgaagctccgaacacaaatacccgcagaaatgctagcaagcattgacctgaagtatttcaatgaatcaacaaggaagaaaattgagaaaataaggcctcttctaatagatggcacagcatcattgagccctgggatgatgatgggcatgttcaacatgctaagtacggttttaggagtctcgatactgaatcttgggcaaaagaaatacaccaagacaacatactggtgggatgggctccaatcctccgacgattttgccctcatagtgaatgcaccaaatcatgagggaatacaagcaggagtggatagattctacaggacctgcaagttagtgggaatcaacatgagcaaaaagaagtcctatataaataaaacagggacatttgaattcacaagctttttttatcgatatggatttgtggctaattttagcatggagcttcccagttttggagtgtctggaataaacgagtcagctgatatgagcattggagtaacagtgataaagaacaacatgataaacaatgaccttggaccagcaacagcccagatggctctccaattgttcatcaaagactacagatatacatataggtgccatagaggagacacacaaattcagacgagaagatcattcgagctaaagaagctgtgggatcaaacccaatcaagggcaggactattggtatcagatgggggaccaaacttatacaatatccggaaccttcacatccctgaagtctgcttaaagtgggagctaatggatgagaattatcagggaagactttgtaaccccctgaatccctttgtcagccataaagaaattgagtctgtaaacaatgctgtagtgatgccagcccatggtccagccaaaagtatggaatatgatgccgttgcaactacacactcctggattcccaagaggaaccgctctattctcaacacaagccaaaggggaattcttgaggatgaacagatgtaccaaaagtgctgcaacttgtttgagaaatttttccctagtagttcatataggagaccgattggaatttctagcatggtggaggccatggtgtctagggcccggattgatgccagaattgacttcgagtctggacggattaagaaggaagagttctctgagatcatgaagatctgttccaccattgaagaactcagacggcaaaaataatgaatttagcttgtccttcatgaaaaaatgccttgtttctact

SEQ ID NO: 7 - DNA, 2341 bp, Influenza virus
agcaaaagcaggcaaaccatttgaatggatgtcaatccgactctacttttcctaaaggttccagcgcaaaatgccataagcaccacattcccctatactggagatcctccatacagccatggaacaggaacaggatacaccatggacacagtcaacagaacgcaccaatattcagaaaaagggaagtggacgacaaacacagaaactggggcaccccaactcaacccgattgatggaccactacctgaggataatgagccaagtggatatgcacaaacagactgtgttctggaggccatggctttccttgaagaatcccacccagggatctttgagaactcatgccttgaaacaatggaagttgttcagcaaacaagggtggataaactaactcaaggtcgccagacttatgattggacattaaacagaaatcaaccggcagcaactgcattagccaacaccatagaagtctttagatcgaatggtctaacagctaatgagtcaggaaggctaatagatttcctaaaggatgtgatggaatcaatggataaagaggaaatagagataacaacacactttcaaagaaaaaggagagtaagagacaacatgaccaagaaaatggtcacacaaagaacaataggaaagaaaaaacaaagagtgaataagagaggctatttaataagagcactgacattgaatacgatgaccaaagatgcagagagaggcaaattaaaaagaagggctattgcaacacccgggatgcaaatgagagggttcgtgtactttgttgaaactttagctaggagcatttgcgaaaagcttgaacagtctggacttccagttgggggtaatgaaaagaaggccaaattggcaaatgttgtgagaaagatgatgactaattcacaagacacagagctttctttcacaatcactggggacaacactaagtggaatgaaaatcaaaatcctcgaatgttcctggcgatgattacatatatcacaaaaaatcaacctgagtggttcagaaacatcctgagcatcgcacccataatgttctcaaacaaaatggcaagactaggaaaagggtacatgttcgagagtaaaagaatgaagctccgaacacaaataccagcagaaatgctagcaagcattgacctgaaatatttcaatgaatcaacaaggaagaaaattgagaaaataaggcctcttctaatagatggcacagcatcattgagccctggaatgatgatgggcatgttcaacatgctaagtacggttttgggagtctcgatactgaatcttggacaaaagaaatacaccaagacaacatactggtgggatgggctccaatcctccgacgattttgccctcatagtgaatgcaccaaatcatgagggaatacaagcaggagtggatagattttacaggacctgcaagttagtgggaatcaacatgagcaaaaagaagtcctatataaataagacagggacatttgaattcacaagctttttttatcgctatggatttgtggctaattttagcatggagctgcccagttttggagtgtctggaataaatgaatcagctgatatgagcattggagtaacagtgataaagaacaacatgataaacaatgaccttggaccagcaacagcccagatggcccttcaattgttcatcaaagactacagatatacatatagatgccatagaggagacacacaaattcagacgagaagatcattcgagctaaagaagctgtgggatcaaacccaatcaaaggcaggactattagtgtcagatggaggaccaaacttatacaatatccggaatcttcacattcctgaagtctgcttaaaatgggagctaatggatgaggattatcggggaagactttgtaatcccctgaatccctttgtcagccataaagagattgagtctgtaaacaatgctgtggtgatgccagcccatggtccagccaaaagcatggaatatgatgccgttgcaactacacactcctggattcccaagaggaaccgctctattctcaacacaagccaaaggggaattcttgaggatgaacagatgtaccagaagtgctgcaacctgttcgagaaatttttccccagtagttcatacaggagaccggttggaatttctagcatggtggaggccatggtgtctagggcccggattgatgccagaattgacttcgagtctggaaggattaagaaagaagagttctctgagatcatgaagatctgttccaccattgaagaactcagacggcaaaaataatgaatttagcttgtccttcatgaaaaaatgccttgtttctact

SEQ ID NO: 8 - DNA, 2233 bp, Influenza virus
agcgaaagcaggtactgatccaaaatggaagattttgtgcgacaatgcttcaatccgatgattgtcgagcttgcggaaaaaacaatgaaagagtatggggaggacctgaaaatcgaaacaaacaaatttgcagcaatatgcactcacttggaagtatgcttcatgtattcagattttcacttcatcaatgagcaaggcgagtcaataatcgtagaacttggtgatccaaatgcacttttgaagcacagatttgaaataatcgagggaagagatcgcacaatggcctggacagtagtaaacagtatttgcaacactacaggggctgagaaaccaaagtttctaccagatttgtatgattacaaggagaatagattcatcgaaattggagtaacaaggagagaagttcacatatactatctggaaaaggccaataaaattaaatctgagaaaacacacatccacattttctcgttcactggggaagaaatggccacaaaggcagactacactctcgatgaagaaagcagggctaggatcaaaaccagactattcaccataagacaagaaatggccagcagaggcctctgggattcctttcgtcagtccgagagaggagaagagacaattgaagaaaggtttgaaatcacaggaacaatgcgcaagcttgccgaccaaagtctcccgccgaacttctccagccttgaaaattttagagcctatgtggatggattcgaaccgaacggctacattgagggcaagctgtctcaaatgtccaaagaagtaaatgctagaattgaaccttttttgaaaacaacaccacgaccacttagacttccgaatgggcctccctgttctcagcggtccaaattcctgctgatggatgccttaaaattaagcattgaggacccaagtcatgaaggagagggaataccgctatatgatgcaatcaaatgcatgagaacattctttggatggaaggaacccaatgttgttaaaccacacgaaaagggaataaatccaaattatcttctgtcatggaagcaagtactggcagaactgcaggacattgagaatgaggagaaaattccaaagactaaaaatatgaagaaaacaagtcagctaaagtgggcacttggtgagaacatggcaccagaaaaggtagactttgacgactgtaaagatgtaggtgatttgaagcaatatgatagtgatgaaccagaattgaggtcgctagcaagttggattcagaatgagtttaacaaggcatgcgaactgacagattcaagctggatagagctcgatgagattggagaagatgtggctccaattgaacacattgcaagcatgagaaggaattatttcacatcagaggtgtctcactgcagagccacagaatacataatgaagggggtgtacatcaatactgccttgcttaatgcatcttgtgcagcaatggatgatttccaattaattccaatgataagcaagtgtagaactaaggagggaaggcgaaagaccaacttgtatggtttcatcataaaaggaagatcccacttaaggaatgacaccgacgtggtaaactttgtgagcatggagttttctctcactgacccaagacttgaaccacataaatgggagaagtactgtgttcttgagataggagatatgcttataagaagtgccataggccaggtttcaaggcccatgttcttgtatgtgagaacaaatggaacctcaaaaattaaaatgaaatggggaatggagatgaggcgttgcctcctccagtcacttcaacaaattgagagtatgattgaagctgagtcctctgtcaaagagaaagacatgaccaaagagttctttgagaacaaatcagaaacatggcccattggagagtcccccaaaggagtggaggaaagttccattgggaaggtctgcaggactttattagcaaagtcggtattcaacagcttgtatgcatctccacaactagaaggattttcagctgaatcaagaaaactgcttcttatcgttcaggctcttagggacaaccttgaacctgggacctttgatcttggggggctatatgaagcaattgaggagtgcctgattaatgatccctgggttttgcttaatgcttcttggttcaactccttccttacacatgcattgagttagttgtggcagtgctactatttgctatccatactgtccaaaaaagtaccttgtttctact

SEQ ID NO: 9 - DNA, 2233 bp, Influenza virus
agcaaaagcaggtactgattcgaaatggaagattttgtgcgacaatgcttcaacccgatgattgtcgaacttgcagaaaaaacaatgaaagagtatggagaggatctgaaaattgaaacaaacaaatttgcagcaatatgcacccacttggaggtatgtttcatgtattcagattttcatttcatcaatgaacaaggcgaatcaataatggtagaacttgatgatccaaatgcactgttaaagcacagattcgaaataatcgaggggagagacagaacaatggcctggacagtagtaaacagtatctgcaacactactggagctgaaaaaccgaagtttctaccagatttgtatgattacaaggagaacagattcatcgaaattggagtgacaagaagagaagtccacatatattaccttgaaaaggccactaaaattaaatctgagaacacacacattcacattttctcattcactggggaggaaatggccacaaaggcagactacactctcgacgaggaaagcagggctaggattaaaaccaggctatttaccataagacaagaaatggccaacagaggcctctgggattcctttcgtcagtccgaaagaggcgaagaaacaattgaagaaaaatttgaaatctcaggaactatgcgtaggcttgccgaccaaagtctcccaccgaacttctcctgccttgagaattttagagcctatgtggatggattcgaaccgaacggctgcattgagggcaagctttctcaaatgtccaaagaagtgaatgccaaaattgaaccttttctgaagacaacaccaagaccaatcaaacttcctaatggacctccttgttatcagcggtccaaattcctcctgatggatgctttgaaattgagcattgaagacccaagtcacgaaggagaagggattccattatatgatgcgatcaagtgcataaaaacattctttggatggaaagaaccttatatagtcaaaccacacgaaaagggaataaattcaaattacctgctgtcatggaagcaagtattgtcagaattgcaggacattgaaaatgaggagaagatcccaaggactaaaaacatgaagaaaacgagtcaactaaagtgggctcttggtgaaaacatggcaccagagaaagtagactttgacaactgcagagacataagcgatttgaagcaatatgatagtgacgaacctgaattaaggtcactttcaagctggatacagaatgagttcaacaaggcctgcgagctaactgattcaatctggatagagctcgatgaaattggagaggacgtagccccaattgagtacattgcaagcatgaggaggaattatttcacagcagaggtgtcccattgtagagccactgagtacataatgaagggggtatacattaatactgccctgctcaatgcatcctgtgcagcaatggacgattttcaattaatccccatgataagcaagtgcagaactaaagagggaaggcgaaaaaccaatttatatggattcatcataaagggaagatctcatttaaggaatgacacagatgtggtaaactttgtgagcatggaattttctctcactgacccgagactagagccacataaatgggagaaatactgtgtccttgagataggagatatgttactaagaagtgccataggccaaatttcaaggcctatgttcttgtatgttaggacaaacggaacatcaaaggtcaaaatgaaatggggaatggagatgagacgttgcctccttcagtcactccagcagatcgagagcatgattgaagccgagtcctcgattaaagagaaagacatgaccaaagagttttttgagaataaatcagaagcgtggcccattggggagtcccccaagggagtggaagaaggttccattgggaaagtctgtaggactctattggctaagtcagtgttcaatagcctgtatgcatcaccacaattggaaggattttcagcggagtcaagaaaactgcttcttgttgttcaggctcttagggacaacctcgaacctgggacctttgatctcggggggctatatgaagcaattgaggagtgcctgattaatgatccctgggttttgctcaatgcatcttggttcaactccttcctgacacatgcattaaaatagttatggcagtgctactatttgttatccgtactgtccaaaaaagtaccttgtttctact

SEQ ID NO: 10 - DNA, 2233 bp, Influenza virus
agcaaaagcaggtactgattcgaaatggaagattttgtgcgacaatgcttcaacccgatgattgtcgaacttgcagaaaaggcaatgaaagagtatggagaggatctgaaaattgaaacaaacaaatttgcagcaatatgcactcacttggaggtatgtttcatgtattcagattttcatttcatcaatgaacaaggtgaatcaatagtggtagaacttgacgatccaaatgcactgttaaagcacagatttgaaataatagaggggagagacagaacgatggcctggacagtagtaaacagtatctgcaacactactggagctgagaaaccgaagtttctgccagatttgtatgattacaaggagaacagattcatcgaaattggagtaacaaggagagaagtccacatatattaccttgaaaaggccaataaaattaaatctgagaatacacacatccacattttctcattcactggggaggaaatggccacaaaggcagactacactctcgacgaggaaagcagggctaggattaagaccaggctatttaccataagacaagaaatggccaacagaggcctctgggattcctttcgtcagtccgaaagaggcgaagagacaattgaagaaaaatttgaaatctcaggaactatgcgcaggcttgccgaccaaagcctcccgccgaacttctcctgccttgagaattttagagcctatgtagatggattcgaaccgaacggctgcattgagggcaagctttctcaaatgtccaaagaagtgaatgccaaaattgaaccttttctgaagacaacaccaagaccaatcaaacttccgaatggacctccttgttatcagcggtccaaattccttctgatggatgctttaaaattaagcattgaagacccaagtcatgaaggagaagggataccactatatgatgcgatcaagtgcataagaacattctttggatggaaagaaccctatatagtcaaaccacacgaaaagggaataaattcaaattacctgctgtcatggaagcaagtactggcagaattgcaggacattgaaactgaggagaagattccaagaactaaaaacatgaagaaaacgagtcaactaaagtgggctcttggtgaaaacatggcaccagagaaagtagactttgacaactgcagagacataagcgatttgaagcaatatgatagtgacgaacctgaattgaggtcactttcaagctggatacagaatgagttcaacaaggcatgcgagctgactgattcaatctggatagagctcgatgaaattggagaagacatagccccaattgagtacattgcaagcatgaggaggaattatttcacagcagaggtgtcccactgcagagccactgagtacataatgaagggggtatacattaatactgccttgctcaatgcatcctgtgcagcaatggacgattttcaactaattcccatgataagcaagtgcagaacaaaagagggaaggcgaaaaaccaatttatatggattcatcataaaagggagatctcacttaaggaatgacacagatgtggtaaactttgtgagcatggagttttctctcactgacccgaggcttgagccacataaatgggagaaatactgtgtccttgagataggagatatgttactaagaagtgccataggccaaatgtcaaggcctatgttcttgtatgtgaggacaaatggaacatcaaagatcaaaatgaaatggggaatggagatgagacgttgcctccttcagtcactccagcagatcgagagcatgattgaagccgagtcctcggttaaagagaaagacatgaccaaagagttttttgagaataaatcagaagcatggcccattggggagtcccccaagggagtggaagaaggttccattgggaaagtttgtaggactttgttggctaagtcggtgttcaatagcctgtatgcatctccacaattagaaggattttcagcggagtcaagaaaactgctccttgttgttcaggctcttagggacaaccttgaacctgggacctttgatcttggggggctatatgaagcaattgaggagtgcctgattaatgatccctgggttttgctcaatgcgtcttggttcaactccttcctgaaacatgcattaaaatagttatggcagtgctactatttgttatccatactgtccaaaaaagtaccttgtttctact

SEQ ID NO: 11 - DNA, 31 bp, Artificial Sequence
  Primer
atggtctctactgatggtgagcaagggcgag

SEQ ID NO: 12 - DNA, 34 bp, Artificial Sequence
  Primer
atgaagacaatctcttacttgtacagctcgtcca

SEQ ID NO: 13 - DNA, 19 bp, Artificial Sequence
  Primer
ggacacgctgaacttgtgg

SEQ ID NO: 14 - DNA, 22 bp, Artificial Sequence
  Primer
agataagaggataatggaaatg

SEQ ID NO: 15 - DNA, 22 bp, Artificial Sequence
  Primer
atatggtccackgtggtttttg

SEQ ID NO: 16 - DNA, 20 bp, Artificial Sequence
  Primer
ggagaagactgaggggattc

SEQ ID NO: 17 - DNA, 20 bp, Artificial Sequence
  Primer
tccatggtgtatcctgttcc

SEQ ID NO: 18 - DNA, 20 bp, Artificial Sequence
  Primer
tgatttcgaatctggaagga

SEQ ID NO: 19 - DNA, 21 bp, Artificial Sequence
  Primer
tgagtgcatattgctgcaaat

SEQ ID NO: 20 - DNA, 20 bp, Artificial Sequence
  Primer
ttcttatcgttcaggctctt

SEQ ID NO: 21 - DNA, 22 bp, Artificial Sequence
  Primer
tccagtatggttttgayttccr

SEQ ID NO: 22 - DNA, 20 bp, Artificial Sequence
  Primer
tggactagtgsgagcatsat

SEQ ID NO: 23 - DNA, 20 bp, Artificial Sequence
  Primer
tcccaggcggtctcccatcc

SEQ ID NO: 24 - RNA, 395 nt, Influenza virus
agcgaaagcaggucaaauauauucaauauggaaagaauaaaagaacuaagaaaucuaaugucgcagucucgcacccgcgagauacucacaaaaaccaccguggaccauauggccauaaucaagaaguacacaucaggaagacaggagaagacugaggggauuccucauucugggcaaagaggacaagagauaugggccagcacuaagcaucaaugaacugagcaaccuugcgaaaggagagaaggcuaaugugcuaauugggcaaggggaugugguguugguaaugaaacggaaacgggacucuagcauacuuacugacagccagacagcgaccaaaagaauucggauggccaucaauuagugucgaauaguuuaaaaacgaccuuguuucuacu

SEQ ID NO: 25 - protein, 62 aa, Influenza virus
MERIKELRNLMSQSRTREILTKTTVDHMAIIKKYTSGRQEKTEGIPHSGQRGQEIWASTKHQ